European Patent Specification EP 3 647 414 B1, published August 7, 2024. Title: GLUCOSE OXIDASE CNGODA AND GENE AND APPLICATION THEREOF. Applicant: Feed Research Institute, Chinese Academy of Agricultural Sciences. The sequence listing filed with the application follows.

SEQUENCE LISTING (4 sequences)

SEQ ID NO: 1 - protein, 613 aa, Cladosporiumneopsychrotolerns SL-16 strain
MHSIHFLAAFLAAVSEALPNQTRADKAHAITTNVDQVSNKTFDYIVCGGGLTGLVVASRLSEDPNISVLVIENGEDDHEDPRVNDVRTYGEAFKSDLDYNLTSTPVPWQNDTGLLLVAGRTLGGSGSLNGASWTKGDRTQYDLLPVLSGDDSWSFDALNEIMLGIEEFHEPTEEQIAKGAQYADEYHGRDGVVQVSFPAGMFGGIQLSALEASTLVWKGLKLVADFAAGVTSGATIIPNMVEPNDSQNRSSPFTVYAKHQTQERSNFLILTGHRVTSINWRNGTGMVADGVTFQACRECEVHTATTKREVLLAAGSLQSPQLLELSGVGDPEVLAAAYVPLKLCSPNVGKNMQEQTKNTLWFDPISTDFDGSGPPNAVAFPDVHQLFKNDSASIYKSIISSLEGYSQNLTAAGIVTNATATRLILEAQVNNLWKDNAGAAEIFFVTSPTTGQVGIDLWNLIVLSRGYVHITSNSSWDHPQIEPSYFGHPFDLEIQLAATKQSREVSQTEPLASLISAETFPGFDEVPQNATDDVWEQWVKETFTSVWHYIATLGMMKEELGGVVDSRLKVYGIENVRAVDASVLPIQLSAHLSSSLYGIAEKAAMMIKEDQGH

SEQ ID NO: 2 - protein, 596 aa, Cladosporiumneopsychrotolerns SL-16 strain
LPNQTRADKAHAITTNVDQVSNKTFDYIVCGGGLTGLVVASRLSEDPNISVLVIENGEDDHEDPRVNDVRTYGEAFKSDLDYNLTSTPVPWQNDTGLLLVAGRTLGGSGSLNGASWTKGDRTQYDLLPVLSGDDSWSFDALNEIMLGIEEFHEPTEEQIAKGAQYADEYHGRDGVVQVSFPAGMFGGIQLSALEASTLVWKGLKLVADFAAGVTSGATIIPNMVEPNDSQNRSSPFTVYAKHQTQERSNFLILTGHRVTSINWRNGTGMVADGVTFQACRECEVHTATTKREVLLAAGSLQSPQLLELSGVGDPEVLAAAYVPLKLCSPNVGKNMQEQTKNTLWFDPISTDFDGSGPPNAVAFPDVHQLFKNDSASIYKSIISSLEGYSQNLTAAGIVTNATATRLILEAQVNNLWKDNAGAAEIFFVTSPTTGQVGIDLWNLIVLSRGYVHITSNSSWDHPQIEPSYFGHPFDLEIQLAATKQSREVSQTEPLASLISAETFPGFDEVPQNATDDVWEQWVKETFTSVWHYIATLGMMKEELGGVVDSRLKVYGIENVRAVDASVLPIQLSAHLSSSLYGIAEKAAMMIKEDQGH

SEQ ID NO: 3 - DNA, 1842 bp, Cladosporiumneopsychrotolerns SL-16
atgcattcgattcatttcctagctgctttcctggctgcagtctctgaagctcttcccaatcaaacgcgagctgacaaagcccatgccatcactacaaacgtcgaccaggtctcaaacaaaactttcgactacatagtctgcggcggaggcttgacaggcctggtcgtcgcaagtcggttgtcagaagacccaaatatatctgttctcgtcattgagaacggagaggacgaccacgaagaccctcgcgtgaacgacgtgagaacctacggagaagccttcaaatccgacctcgactacaacctcacatcaaccccagtaccatggcagaacgacacaggtctacttcttgtggctggcaggacacttggtggaagtggcagtctcaatggtgccagctggactaaaggcgacaggacgcagtatgatttgctcccggtcttgagcggcgatgactcgtggtccttcgatgctttgaacgagatcatgctaggcattgaagagttccacgaaccgactgaagaacagattgccaaaggtgcacagtatgcagacgaataccatggccgtgacggagttgtccaagtctccttcccagctggcatgttcggcggcattcaactttcggctttggaagcttccactctcgtctggaagggcctgaaacttgtcgcggactttgcagccggagtgacaagtggtgcgaccatcatcccaaacatggttgagccaaacgactcccaaaatcggtcttccccattcacggtctatgccaagcaccagactcaggaacgcagcaacttcttgatcttgacaggacaccgtgtgacatccatcaactggcgcaacggcactggcatggtagctgatggtgtcacatttcaagcatgccgcgaatgcgaggtacacacagccacgacaaagcgagaagtactgctcgccgcgggctcgttgcagagcccacagcttctcgagctctctggcgtgggtgatcctgaggtcttggccgccgcatatgttcctctgaagctgtgttctcccaatgttggtaagaacatgcaggaacagaccaaaaacactctctggttcgaccccatcagcaccgatttcgatggttccggacctccaaacgcagttgctttcccggacgtccaccaactgttcaaaaatgacagtgcaagcatttacaaatctatcatttccagcctcgaaggatactcacaaaacctgaccgccgccggcatcgtcacaaacgccacagcaacacgcctcatccttgaagcacaagtcaacaacctctggaaagataacgccggagcagcagagatcttcttcgtgacttcacccaccacaggccaagttggcattgatctctggaacctcatcgtcctgtcccgaggctacgtgcacatcacttcgaactcctcctgggaccacccccaaatcgagccctcctacttcggccaccctttcgaccttgagattcagctcgcagccaccaagcaatcacgcgaagtctcccaaacagaacctctcgcctcgctcatcagcgccgagacatttcctggtttcgatgaagtgccgcaaaatgccacagacgatgtgtgggagcagtgggttaaggagacgttcacatctgtttggcactacatagctacattgggcatgatgaaagaggaattgggtggtgttgtggacagcaggctgaaggtatatggcattgagaatgtacgagcggtggatgctagtgtgctgccgatccagctttcggcgcacttgagctcttcgctgtacggcattgcggagaaggctgctatgatgattaaggaagatcagggacattga

SEQ ID NO: 4 - DNA, 1791 bp, Cladosporiumneopsychrotolerns SL-16
cttcccaatcaaacgcgagctgacaaagcccatgccatcactacaaacgtcgaccaggtctcaaacaaaactttcgactacatagtctgcggcggaggcttgacaggcctggtcgtcgcaagtcggttgtcagaagacccaaatatatctgttctcgtcattgagaacggagaggacgaccacgaagaccctcgcgtgaacgacgtgagaacctacggagaagccttcaaatccgacctcgactacaacctcacatcaaccccagtaccatggcagaacgacacaggtctacttcttgtggctggcaggacacttggtggaagtggcagtctcaatggtgccagctggactaaaggcgacaggacgcagtatgatttgctcccggtcttgagcggcgatgactcgtggtccttcgatgctttgaacgagatcatgctaggcattgaagagttccacgaaccgactgaagaacagattgccaaaggtgcacagtatgcagacgaataccatggccgtgacggagttgtccaagtctccttcccagctggcatgttcggcggcattcaactttcggctttggaagcttccactctcgtctggaagggcctgaaacttgtcgcggactttgcagccggagtgacaagtggtgcgaccatcatcccaaacatggttgagccaaacgactcccaaaatcggtcttccccattcacggtctatgccaagcaccagactcaggaacgcagcaacttcttgatcttgacaggacaccgtgtgacatccatcaactggcgcaacggcactggcatggtagctgatggtgtcacatttcaagcatgccgcgaatgcgaggtacacacagccacgacaaagcgagaagtactgctcgccgcgggctcgttgcagagcccacagcttctcgagctctctggcgtgggtgatcctgaggtcttggccgccgcatatgttcctctgaagctgtgttctcccaatgttggtaagaacatgcaggaacagaccaaaaacactctctggttcgaccccatcagcaccgatttcgatggttccggacctccaaacgcagttgctttcccggacgtccaccaactgttcaaaaatgacagtgcaagcatttacaaatctatcatttccagcctcgaaggatactcacaaaacctgaccgccgccggcatcgtcacaaacgccacagcaacacgcctcatccttgaagcacaagtcaacaacctctggaaagataacgccggagcagcagagatcttcttcgtgacttcacccaccacaggccaagttggcattgatctctggaacctcatcgtcctgtcccgaggctacgtgcacatcacttcgaactcctcctgggaccacccccaaatcgagccctcctacttcggccaccctttcgaccttgagattcagctcgcagccaccaagcaatcacgcgaagtctcccaaacagaacctctcgcctcgctcatcagcgccgagacatttcctggtttcgatgaagtgccgcaaaatgccacagacgatgtgtgggagcagtgggttaaggagacgttcacatctgtttggcactacatagctacattgggcatgatgaaagaggaattgggtggtgttgtggacagcaggctgaaggtatatggcattgagaatgtacgagcggtggatgctagtgtgctgccgatccagctttcggcgcacttgagctcttcgctgtacggcattgcggagaaggctgctatgatgattaaggaagatcagggacattga